European Patent Specification EP 3 601 596 B1, published December 3, 2025. Title: STRAND-SPECIFIC DETECTION OF BISULFITE-CONVERTED DUPLEXES. Applicant: The Johns Hopkins University. The sequence listing filed with the application follows.

SEQUENCE LISTING (48 sequences)

SEQ ID NO: 1 - DNA, 65 bp, Artificial Sequence
  Chemically modified sequences
  misc_feature (1)...(65): n = A,T,C or G
cgacgtaaaacgacggccagtnnnnnnnnnnnnnnggattagttggattgttagtgtgttttttt

SEQ ID NO: 2 - DNA, 77 bp, Artificial Sequence
  Chemically modified sequences
  misc_feature (1)...(77): n = A,T,C or G
cgacgtaaaacgacggccagtnnnnnnnnnnnnnncaaaataattctaaattaactaaattatcaatacacttttcc

SEQ ID NO: 3 - DNA, 78 bp, Artificial Sequence
  Chemically modified sequences
  misc_feature (1)...(78): n = A,T,C or G
cgacgtaaaacgacggccagtnnnnnnnnnnnnnnagtattgagaaattgataaatgtatgaatagtattaaattaga

SEQ ID NO: 4 - DNA, 73 bp, Artificial Sequence
  Chemically modified sequences
  misc_feature (1)...(73): n = A,T,C or G
cgacgtaaaacgacggccagtnnnnnnnnnnnnnncaaaaaattaacaaacatataaacaacattaaaccaaa

SEQ ID NO: 5 - DNA, 83 bp, Artificial Sequence
  Chemically modified sequences
  misc_feature (1)...(83): n = A,T,C or G
cgacgtaaaacgacggccagtnnnnnnnnnnnnnnatttgttttgatgtaataaatatgtatatattattatattagtttgtt

SEQ ID NO: 6 - DNA, 76 bp, Artificial Sequence
  Chemically modified sequences
  misc_feature (1)...(76): n = A,T,C or G
cgacgtaaaacgacggccagtnnnnnnnnnnnnnnccaatataataaatatacacatatcattacaccaattcatc

SEQ ID NO: 7 - DNA, 71 bp, Artificial Sequence
  Chemically modified sequences
  misc_feature (1)...(71): n = A,T,C or G
cgacgtaaaacgacggccagtnnnnnnnnnnnnnngggaatttaaagtatatgaatttgtttttttgttgt

SEQ ID NO: 8 - DNA, 67 bp, Artificial Sequence
  Chemically modified sequences
  misc_feature (1)...(67): n = A,T,C or G
cgacgtaaaacgacggccagtnnnnnnnnnnnnnnactcaaaatacataaacttatcttcccatcat

SEQ ID NO: 9 - DNA, 74 bp, Artificial Sequence
  Chemically modified sequences
  misc_feature (1)...(74): n = A,T,C or G
cgacgtaaaacgacggccagtnnnnnnnnnnnnnngaagataagtttatgtattttgagtttttttagttgtta

SEQ ID NO: 10 - DNA, 69 bp, Artificial Sequence
  Chemically modified sequences
  misc_feature (1)...(69): n = A,T,C or G
cgacgtaaaacgacggccagtnnnnnnnnnnnnnncaaattcatatactttaaattccctcaaccatta

SEQ ID NO: 11 - DNA, 64 bp, Artificial Sequence
  Chemically modified sequences
  misc_feature (1)...(64): n = A,T,C or G
cgacgtaaaacgacggccagtnnnnnnnnnnnnnnggagaaaagtattggttggttttgttttt

SEQ ID NO: 12 - DNA, 80 bp, Artificial Sequence
  Chemically modified sequences
  misc_feature (1)...(80): n = A,T,C or G
cgacgtaaaacgacggccagtnnnnnnnnnnnnnnactaaccttaaaatttaaaaaaaaatatcaattaactttatcttt

SEQ ID NO: 13 - DNA, 56 bp, Artificial Sequence
  Chemically modified sequences
  misc_feature (1)...(56): n = A,T,C or G
cgacgtaaaacgacggccagtnnnnnnnnnnnnnngtgtgtagggtgaagtgtgag

SEQ ID NO: 14 - DNA, 80 bp, Artificial Sequence
  Chemically modified sequences
  misc_feature (1)...(80): n = A,T,C or G
cgacgtaaaacgacggccagtnnnnnnnnnnnnnnccaaaactaaataaaactccaaatatatataaaacaaaatataaa

SEQ ID NO: 15 - DNA, 66 bp, Artificial Sequence
  Chemically modified sequences
  misc_feature (1)...(66): n = A,T,C or G
cgacgtaaaacgacggccagtnnnnnnnnnnnnnnggagaatgttagtttgagttaggtttttttg

SEQ ID NO: 16 - DNA, 74 bp, Artificial Sequence
  Chemically modified sequences
  misc_feature (1)...(74): n = A,T,C or G
cgacgtaaaacgacggccagtnnnnnnnnnnnnnncaaaaaataaaaaatatcaatctaaatcaaacccttcta

SEQ ID NO: 17 - DNA, 71 bp, Artificial Sequence
  Chemically modified sequences
cacacaggaaacagctatgaccatgattataaaaaactttaaaatactataaatataactcaccaattaac

SEQ ID NO: 18 - DNA, 62 bp, Artificial Sequence
  Chemically modified sequences
cacacaggaaacagctatgaccatgagttttaaagtattgtagatgtggtttgttaattaat

SEQ ID NO: 19 - DNA, 58 bp, Artificial Sequence
  Chemically modified sequences
cacacaggaaacagctatgaccatgcattaactcatcctaaattataacaatcaccaa

SEQ ID NO: 20 - DNA, 70 bp, Artificial Sequence
  Chemically modified sequences
cacacaggaaacagctatgaccatggaaaagagaatgtattaatttattttgaattgtagtaattattaa

SEQ ID NO: 21 - DNA, 63 bp, Artificial Sequence
  Chemically modified sequences
cacacaggaaacagctatgaccatgcaactaaaacttatcaaacccttttataaaaatcttaa

SEQ ID NO: 22 - DNA, 69 bp, Artificial Sequence
  Chemically modified sequences
cacacaggaaacagctatgaccatgttattatagttagaatttattaaatttttttgtgaagattttga

SEQ ID NO: 23 - DNA, 70 bp, Artificial Sequence
  Chemically modified sequences
cacacaggaaacagctatgaccatgtttaacaatttaacaattaaaaacatttcctataaaataatacta

SEQ ID NO: 24 - DNA, 64 bp, Artificial Sequence
  Chemically modified sequences
cacacaggaaacagctatgaccatgagtttgatagttaaaggtattttttgtgaaataatattg

SEQ ID NO: 25 - DNA, 66 bp, Artificial Sequence
  Chemically modified sequences
cacacaggaaacagctatgaccatgttttaatctatccttattttaaatatttctcccaataaaaa

SEQ ID NO: 26 - DNA, 69 bp, Artificial Sequence
  Chemically modified sequences
cacacaggaaacagctatgaccatgagtttttaatttgtttttattttggatattttttttaatgaaag

SEQ ID NO: 27 - DNA, 73 bp, Artificial Sequence
  Chemically modified sequences
cacacaggaaacagctatgaccatgcaaaaaaaataaaaaataaaaatctatataatcaaaaaatcaataaca

SEQ ID NO: 28 - DNA, 60 bp, Artificial Sequence
  Chemically modified sequences
cacacaggaaacagctatgaccatgaaatggaagtttatgtgattaagaaattgatagta

SEQ ID NO: 29 - DNA, 60 bp, Artificial Sequence
  Chemically modified sequences
cacacaggaaacagctatgaccatgccactatacctatacaataccaataataacaacaa

SEQ ID NO: 30 - DNA, 58 bp, Artificial Sequence
  Chemically modified sequences
cacacaggaaacagctatgaccatggttgtatttgtgtaatgttagtgatgatgataa

SEQ ID NO: 31 - DNA, 54 bp, Artificial Sequence
  Chemically modified sequences
cacacaggaaacagctatgaccatgctcatataatatcatctctcctccctact

SEQ ID NO: 32 - DNA, 69 bp, Artificial Sequence
  Chemically modified sequences
cacacaggaaacagctatgaccatggtatagatttttttatttatgtgatgttattttttttttttgtt

SEQ ID NO: 33 - DNA, 158 bp, Artificial Sequence
  Chemically modified sequences
ggattagttggattgttagtgtgttttttttaatattatttgttttaattattattagtttgtatttagttattttatattagtaagaatttgttggaaattagtaattagggttaattggtgagttatatttatagtattttaaagttttttataat

SEQ ID NO: 34 - DNA, 161 bp, Artificial Sequence
  Chemically modified sequences
caaaataattctaaattaactaaattatcaatacacttttcccaacaccacctactccaaccaccaccaatttatactcaatcatttcacaccaacaaaaacctattaaaaaccaataatcaaaattaattaacaaaccacatctacaatactttaaaact

SEQ ID NO: 35 - DNA, 150 bp, Artificial Sequence
  Chemically modified sequences
agtattgagaaattgataaatgtatgaatagtattaaattagattttatttagttgagaaagatgagagattaatatttgatgtaagtatttgaaatggaattttatatatgaataattggtgattgttataatttaggatgagttaatg

SEQ ID NO: 36 - DNA, 157 bp, Artificial Sequence
  Chemically modified sequences
caaaaaattaacaaacatataaacaacattaaaccaaaccttatccaactaaaaaaaacaaaaaaccaatacttaatataaatatttaaaataaaatcctatacataaataattaataattactacaattcaaaataaattaatacattctcttttc

SEQ ID NO: 37 - DNA, 145 bp, Artificial Sequence
  Chemically modified sequences
atttgttttgatgtaataaatatgtatatattattatattagtttgtttttttttagttttatagtgaattgttgtaatatgattgttatttttatttagttattggttaagatttttataaaagggtttgataagttttagttg

SEQ ID NO: 38 - DNA, 144 bp, Artificial Sequence
  Chemically modified sequences
ccaatataataaatatacacatatcattacaccaattcatccctttccaactttacaataaattactacaacataattatcatcttcacttaaccattaatcaaaatcttcacaaaaaaatttaataaattctaactataataa

SEQ ID NO: 39 - DNA, 162 bp, Artificial Sequence
  Chemically modified sequences
gggaatttaaagtatatgaatttgtttttttgttgtgtgggttttgaattggaggaatatatttttatttttagttggtagattataaattgaggatttgtatggttaaatatatattagtattattttataggaaatgtttttaattgttaaattgttaaa

SEQ ID NO: 40 - DNA, 152 bp, Artificial Sequence
  Chemically modified sequences
actcaaaatacataaacttatcttcccatcatataaatcctaaattaaaaaaatatatcttcacctttaactaacaaaccacaaactaaaaatctacataattaaatacataccaatattatttcacaaaaaatacctttaactatcaaact

SEQ ID NO: 41 - DNA, 152 bp, Artificial Sequence
  Chemically modified sequences
gaagataagtttatgtattttgagtttttttagttgttatttgtgtgtggtgatattaaagtagagtttttttataaatagaataagatgttaaaaaaggtttgtattttatttttattgggagaaatatttaaaataaggatagattaaaa

SEQ ID NO: 42 - DNA, 150 bp, Artificial Sequence
  Chemically modified sequences
caaattcatatactttaaattccctcaaccattacctatatataataatatcaaaataaaattcttccacaaacaaaacaaaatactaaaaaaaatttatactttactttcattaaaaaaaatatccaaaataaaaacaaattaaaaact

SEQ ID NO: 43 - DNA, 157 bp, Artificial Sequence
  Chemically modified sequences
ggagaaaagtattggttggttttgtttttatttgttttgttaagattattttttgttaaagtaagtattagatattttttgttattatttgtatgttttatattgtaaatgttattgattttttgattatatagatttttattttttattttttttg

SEQ ID NO: 44 - DNA, 160 bp, Artificial Sequence
  Chemically modified sequences
actaaccttaaaatttaaaaaaaaatatcaattaactttatctttatttactttatcaaaatcattttttattaaaataaatactaaatattccttatcattatctacacactctatactacaaatactatcaatttcttaatcacataaacttccattt

SEQ ID NO: 45 - DNA, 143 bp, Artificial Sequence
  Chemically modified sequences
gtgtgtagggtgaagtgtgagtttattttgttagttagtgataggtaggggtggggggtttgttgaggattttttagtttgatgatgttgatgaatttaggttttagattgttgttattattggtattgtataggtatagtgg

SEQ ID NO: 46 - DNA, 165 bp, Artificial Sequence
  Chemically modified sequences
ccaaaactaaataaaactccaaatatatataaaacaaaatataaatctaccttactaaccaataacaaacaaaaacaaaaaacccatcaaaaactctccaacttaacaatactaataaatccaaactccaaattatcatcatcactaacattacacaaatacaac

SEQ ID NO: 47 - DNA, 133 bp, Artificial Sequence
  Chemically modified sequences
ggagaatgttagtttgagttaggtttttttgttttgaatatgagttttttatggtgggaggtagattgattttttttggattttaggtggttgtaggagatagaagtagggaggagagatgatattatatgag

SEQ ID NO: 48 - DNA, 156 bp, Artificial Sequence
  Chemically modified sequences
caaaaaataaaaaatatcaatctaaatcaaacccttctatcttaaacataaattttttataacaaaaaataaactaaccctttttaaacttcaaataactataaaaaacaaaaacaaaaaaaaaaaataacatcacataaataaaaaaatctatac